European Patent Specification EP 3 518 948 B1, published April 12, 2023. Title: COMPOSITIONS AND METHODS FOR ENHANCING GROWTH, SPREAD, AND ONCOLYTIC AND IMMUNOTHERAPEUTIC EFFICACY OF ONCOLYTIC RNA VIRUSES. Applicant: Ottawa Hospital Research Institute. The sequence listing filed with the application follows.

SEQUENCE LISTING (40 sequences)

SEQ ID NO: 1 - DNA, 20 bp, Artificial Sequence
  primer
atactcagatgtggcagccg

SEQ ID NO: 2 - DNA, 20 bp, Artificial Sequence
  primer
gatctgccaataccgctgga

SEQ ID NO: 3 - DNA, 20 bp, Artificial Sequence
  primer
agtgcaaggaaccccagtag

SEQ ID NO: 4 - DNA, 20 bp, Artificial Sequence
  primer
agggcttggggcaaattgtt

SEQ ID NO: 5 - DNA, 20 bp, Artificial Sequence
  primer
tgctgaagctcacacccttg

SEQ ID NO: 6 - DNA, 22 bp, Artificial Sequence
  primer
ggaaactgaatctggctgagca

SEQ ID NO: 7 - DNA, 20 bp, Artificial Sequence
  primer
ttccgtcacctgctcagaat

SEQ ID NO: 8 - DNA, 21 bp, Artificial Sequence
  primer
cagcagcaagtgatgcagaga

SEQ ID NO: 9 - DNA, 24 bp, Artificial Sequence
  primer
acccccaataaatataggactgga

SEQ ID NO: 10 - DNA, 20 bp, Artificial Sequence
  primer
gaaggcgcttgtggagaagg

SEQ ID NO: 11 - DNA, 20 bp, Artificial Sequence
  primer
accggaaggaaccatctcac

SEQ ID NO: 12 - DNA, 21 bp, Artificial Sequence
  primer
ggcaaaactgcaccttcacac

SEQ ID NO: 13 - DNA, 20 bp, Artificial Sequence
  primer
gctgcactttggagtgatcg

SEQ ID NO: 14 - DNA, 21 bp, Artificial Sequence
  primer
gagggtttgctacaacatggg

SEQ ID NO: 15 - DNA, 21 bp, Artificial Sequence
  primer
ctgagcctacagcagaggaac

SEQ ID NO: 16 - DNA, 22 bp, Artificial Sequence
  primer
aggtactccttgaatgccactt

SEQ ID NO: 17 - DNA, 23 bp, Artificial Sequence
  primer
cagcatttctactccttccaaga

SEQ ID NO: 18 - DNA, 20 bp, Artificial Sequence
  primer
tggggaagccttgaacaact

SEQ ID NO: 19 - DNA, 20 bp, Artificial Sequence
  primer
gcagtcgtccacaggtcaag

SEQ ID NO: 20 - DNA, 20 bp, Artificial Sequence
  primer
tcttctctgggttggcacac

SEQ ID NO: 21 - DNA, 20 bp, Artificial Sequence
  primer
gcacagacctaacagcaccc

SEQ ID NO: 22 - DNA, 23 bp, Artificial Sequence
  primer
ttggtgacctcactcatgatggc

SEQ ID NO: 23 - DNA, 20 bp, Artificial Sequence
  primer
gcacagacctaacagcaccc

SEQ ID NO: 24 - DNA, 23 bp, Artificial Sequence
  primer
ttggtgacctcactcatgatggc

SEQ ID NO: 25 - DNA, 20 bp, Artificial Sequence
  primer
acagtcagccgcatcttctt

SEQ ID NO: 26 - DNA, 20 bp, Artificial Sequence
  primer
gttaaaagcagccctggtga

SEQ ID NO: 27 - DNA, 21 bp, Artificial Sequence
  primer
cagtgtggagttcgaggaacc

SEQ ID NO: 28 - DNA, 21 bp, Artificial Sequence
  primer
tttgttgcaattggggcttgg

SEQ ID NO: 29 - DNA, 20 bp, Artificial Sequence
  primer
ccatatggagctgacacccc

SEQ ID NO: 30 - DNA, 21 bp, Artificial Sequence
  primer
tcaggaaaatgacacctggct

SEQ ID NO: 31 - DNA, 21 bp, Artificial Sequence
  primer
tcctctctgcaagagacttcc

SEQ ID NO: 32 - DNA, 21 bp, Artificial Sequence
  primer
ggtctgttgggagtggtatcc

SEQ ID NO: 33 - DNA, 21 bp, Artificial Sequence
  primer
cagctgctcaaggcttcctta

SEQ ID NO: 34 - DNA, 20 bp, Artificial Sequence
  primer
caactttgtcgcagccgtta

SEQ ID NO: 35 - DNA, 20 bp, Artificial Sequence
  primer
ctgctgctttgcctacctct

SEQ ID NO: 36 - DNA, 20 bp, Artificial Sequence
  primer
cgagtgacaaacacgactgc

SEQ ID NO: 37 - DNA, 21 bp, Artificial Sequence
  primer
cagtgtggagttcgaggaacc

SEQ ID NO: 38 - DNA, 21 bp, Artificial Sequence
  primer
tttgttgcaattggggcttgg

SEQ ID NO: 39 - DNA, 19 bp, Artificial Sequence
  primer
aggtctcaaacatgatctg

SEQ ID NO: 40 - DNA, 19 bp, Artificial Sequence
  primer
aggtatcctgaccctgaag